European Patent Application EP 4 434 536 A1, published September 25, 2024. Title: Stapled peptide and use thereof. Applicant: MEDSHINE DISCOVERY INC. The sequence listing filed with the application follows.

SEQUENCE LISTING (6 sequences)

SEQ ID NO: 1 - protein, 39 aa, synthetic construct
  VARIANT 2: note = Aib
  VARIANT 39: note = X2
  VARIANT 13: note = X1
  MOD_RES 17: note = 1Lys
  MOD_RES 20: note = 1Lys
YXQGTFTSDYSIXLDKKAQKAFIEYLLEGGPSSGAPPPX

SEQ ID NO: 2 - protein, 39 aa, synthetic construct
  VARIANT 2: note = Aib
  VARIANT 13: note = X1
  MOD_RES 16: note = 1Lys
  MOD_RES 19: note = 1Lys
  VARIANT 20: note = Aib
  VARIANT 39: note = X2
YXQGTFTSDYSIXLDKKAKXAFIEYLLEGGPSSGAPPPX

SEQ ID NO: 3 - protein, 39 aa, synthetic construct
  VARIANT 2: note = Aib
  VARIANT 39: note = X2
  VARIANT 13: note = X1
  MOD_RES 20: note = 1Lys
  MOD_RES 23: note = 1Lys
YXQGTFTSDYSIXLDKKAQKAFKEYLLEGGPSSGAPPPX

SEQ ID NO: 4 - protein, 39 aa, synthetic construct
  VARIANT 2: note = Aib
  VARIANT 39: note = X2
  VARIANT 13: note = X1
  VARIANT 20: note = Aib
  MOD_RES 21: note = 1Lys
  MOD_RES 24: note = 1Lys
YXQGTFTSDYSIXLDKKAQXKFIKYLLEGGPSSGAPPPX

SEQ ID NO: 5 - protein, 39 aa, synthetic construct
  VARIANT 2: note = Aib
  VARIANT 39: note = X2
  VARIANT 13: note = X1
  VARIANT 20: note = Aib
  MOD_RES 25: note = 1Lys
  MOD_RES 28: note = 1Lys
YXQGTFTSDYSIXLDKKAQXAFIEKLLKGGPSSGAPPPX

SEQ ID NO: 6 - protein, 39 aa, synthetic construct
  VARIANT 2: note = Aib
  VARIANT 39: note = X2
  VARIANT 13: note = X1
  VARIANT 20: note = Aib
  MOD_RES 24: note = 1Lys
  MOD_RES 27: note = 1Lys
YXQGTFTSDYSIXLDKKAQXAFIKYLKEGGPSSGAPPPX